European Patent Specification EP 3 538 560 B1, published April 8, 2026. Title: GDNF FUSION POLYPEPTIDES AND METHODS OF USE THEREOF. Applicant: Keros Therapeutics, Inc. The sequence listing filed with the application follows.

SEQUENCE LISTING (37 sequences)

SEQ ID NO: 1 - protein, 211 aa, Homo sapiens
MKLWDVVAVCLVLLHTASAFPLPAGKRPPEAPAEDRSLGRRRAPFALSSDSNMPEDYPDQFDDVMDFIQATIKRLKRSPDKQMAVLPRRERNRQAAAANPENSRGKGRRGQRGKNRGCVLTAIHLNVTDLGLGYETKEELIFRYCSGSCDAAETTYDKILKNLSRNRRLVSDKVGQACCRPIAFDDDLSFLDDNLVYHILRKHSAKRCGCI

SEQ ID NO: 2 - protein, 11 aa, Artificial Sequence
  Synthetic Construct
DICLPRWGCLW

SEQ ID NO: 3 - protein, 246 aa, Homo sapiens
MEWSWVFLFFLSVTTGVHSDKTHTCPPCPAPELLGGPSVFLFPPKPKDTLMISRTPEVTCVVVDVSHEDPEVKFNWYVDGVEVHNAKTKPREEQYNSTYRVVSVLTVLHQDWLNGKEYKCKVSNKALPAPIEKTISKAKGQPREPQVYTLPPSRDELTKNQVSLTCLVKGFYPSDIAVEWESNGQPENNYKTTPPVLDSDGSFFLYSKLTVDKSRWQQGNVFSCSVMHEALHNHYTQKSLSLSPGK

SEQ ID NO: 4 - protein, 3 aa, Artificial Sequence
  Synthetic Construct
GGG

SEQ ID NO: 5 - protein, 5 aa, Artificial Sequence
  Synthetic Construct
GGGGS

SEQ ID NO: 6 - protein, 4 aa, Artificial Sequence
  Synthetic Construct
GGSG

SEQ ID NO: 7 - protein, 4 aa, Artificial Sequence
  Synthetic Construct
SGGG

SEQ ID NO: 8 - protein, 4 aa, Artificial Sequence
  Synthetic Construct
GSGS

SEQ ID NO: 9 - protein, 6 aa, Artificial Sequence
  Synthetic Construct
GSGSGS

SEQ ID NO: 10 - protein, 8 aa, Artificial Sequence
  Synthetic Construct
GSGSGSGS

SEQ ID NO: 11 - protein, 10 aa, Artificial Sequence
  Synthetic Construct
GSGSGSGSGS

SEQ ID NO: 12 - protein, 12 aa, Artificial Sequence
  Synthetic Construct
GSGSGSGSGSGS

SEQ ID NO: 13 - protein, 6 aa, Artificial Sequence
  Synthetic Construct
GGSGGS

SEQ ID NO: 14 - protein, 9 aa, Artificial Sequence
  Synthetic Construct
GGSGGSGGS

SEQ ID NO: 15 - protein, 12 aa, Artificial Sequence
  Synthetic Construct
GGSGGSGGSGGS

SEQ ID NO: 16 - protein, 4 aa, Artificial Sequence
  Synthetic Construct
GGSG

SEQ ID NO: 17 - protein, 4 aa, Artificial Sequence
  Synthetic Construct
GGSG

SEQ ID NO: 18 - protein, 8 aa, Artificial Sequence
  Synthetic Construct
GGSGGGSG

SEQ ID NO: 19 - protein, 12 aa, Artificial Sequence
  Synthetic Construct
GGSGGGSGGGSG

SEQ ID NO: 20 - protein, 5 aa, Artificial Sequence
  Synthetic Construct
GGGGS

SEQ ID NO: 21 - protein, 15 aa, Artificial Sequence
  Synthetic Construct
GGGGSGGGGSGGGGS

SEQ ID NO: 22 - protein, 9 aa, Artificial Sequence
  Synthetic Construct
GGGGAGGGG

SEQ ID NO: 23 - protein, 10 aa, Artificial Sequence
  Synthetic Construct
GENLYFQSGG

SEQ ID NO: 24 - protein, 8 aa, Artificial Sequence
  Synthetic Construct
SACYCELS

SEQ ID NO: 25 - protein, 5 aa, Artificial Sequence
  Synthetic Construct
RSIAT

SEQ ID NO: 26 - protein, 17 aa, Artificial Sequence
  Synthetic Construct
RPACKIPNDLKQKVMNH

SEQ ID NO: 27 - protein, 36 aa, Artificial Sequence
  Synthetic Construct
GGSAGGSGSGSSGGSSGASGTGTAGGTGSGSGTGSG

SEQ ID NO: 28 - protein, 17 aa, Artificial Sequence
  Synthetic Construct
AAANSSIDLISVPVDSR

SEQ ID NO: 29 - protein, 36 aa, Artificial Sequence
  Synthetic Construct
GGSGGGSEGGGSEGGGSEGGGSEGGGSEGGGSGGGS

SEQ ID NO: 30 - protein, 93 aa, Homo sapiens
GPVEVFITETPSQPNSHPIQWNAPQPSHISKYILRWRPKNSVGRWKEATIPGHLNSYTIKGLKPGVVYEGQLISIQQYGHQEVTRFDFTTTST

SEQ ID NO: 31 - protein, 609 aa, Homo sapiens [sequence omitted]

SEQ ID NO: 32 - protein, 380 aa, Artificial Sequence
  Synthetic Construct
MEWSWVFLFFLSVTTGVHSDKTHTCPPCPAPELLGGPSVFLFPPKPKDTLMISRTPEVTCVVVDVSHEDPEVKFNWYVDGVEVHNAKTKPREEQYNSTYRVVSVLTVLHQDWLNGKEYKCKVSNKALPAPIEKTISKAKGQPREPQVYTLPPSRDELTKNQVSLTCLVKGFYPSDIAVEWESNGQPENNYKTTPPVLDSDGSFFLYSKLTVDKSRWQQGNVFSCSVMHEALHNHYTQKSLSLSPGKSPDKQMAVLPRRERNRQAAAANPENSRGKGRRGQRGKNRGCVLTAIHLNVTDLGLGYETKEELIFRYCSGSCDAAETTYDKILKNLSRNRRLVSDKVGQACCRPIAFDDDLSFLDDNLVYHILRKHSAKRCGCI

SEQ ID NO: 33 - protein, 369 aa, Artificial Sequence
  Synthetic Construct
MEWSWVFLFFLSVTTGVHSDKTHTCPPCPAPELLGGPSVFLFPPKPKDTLMISRTPEVTCVVVDVSHEDPEVKFNWYVDGVEVHNAKTKPREEQYNSTYRVVSVLTVLHQDWLNGKEYKCKVSNKALPAPIEKTISKAKGQPREPQVYTLPPSRDELTKNQVSLTCLVKGFYPSDIAVEWESNGQPENNYKTTPPVLDSDGSFFLYSKLTVDKSRWQQGNVFSCSVMHEALHNHYTQKSLSLSPGKGGGNRQAAAANPENSRGKGRRGQRGKNRGCVLTAIHLNVTDLGLGYETKEELIFRYCSGSCDAAETTYDKILKNLSRNRRLVSDKVGQACCRPIAFDDDLSFLDDNLVYHILRKHSAKRCGCI

SEQ ID NO: 34 - protein, 351 aa, Artificial Sequence
  Synthetic Construct
MEWSWVFLFFLSVTTGVHSDKTHTCPPCPAPELLGGPSVFLFPPKPKDTLMISRTPEVTCVVVDVSHEDPEVKFNWYVDGVEVHNAKTKPREEQYNSTYRVVSVLTVLHQDWLNGKEYKCKVSNKALPAPIEKTISKAKGQPREPQVYTLPPSRDELTKNQVSLTCLVKGFYPSDIAVEWESNGQPENNYKTTPPVLDSDGSFFLYSKLTVDKSRWQQGNVFSCSVMHEALHNHYTQKSLSLSPGKGGGGQRGKNRGCVLTAIHLNVTDLGLGYETKEELIFRYCSGSCDAAETTYDKILKNLSRNRRLVSDKVGQACCRPIAFDDDLSFLDDNLVYHILRKHSAKRCGCI

SEQ ID NO: 35 - protein, 344 aa, Artificial Sequence
  Synthetic Construct
MEWSWVFLFFLSVTTGVHSDKTHTCPPCPAPELLGGPSVFLFPPKPKDTLMISRTPEVTCVVVDVSHEDPEVKFNWYVDGVEVHNAKTKPREEQYNSTYRVVSVLTVLHQDWLNGKEYKCKVSNKALPAPIEKTISKAKGQPREPQVYTLPPSRDELTKNQVSLTCLVKGFYPSDIAVEWESNGQPENNYKTTPPVLDSDGSFFLYSKLTVDKSRWQQGNVFSCSVMHEALHNHYTQKSLSLSPGKGGGGCVLTAIHLNVTDLGLGYETKEELIFRYCSGSCDAAETTYDKILKNLSRNRRLVSDKVGQACCRPIAFDDDLSFLDDNLVYHILRKHSAKRCGCI

SEQ ID NO: 36 - protein, 350 aa, Artificial Sequence
  Synthetic Construct
MEWSWVFLFFLSVTTGVHSDKTHTCPPCPAPELLGGPSVFLFPPKPKDTLMISRTPEVTCVVVDVSHEDPEVKFNWYVDGVEVHNAKTKPREEQYNSTYRVVSVLTVLHQDWLNGKEYKCKVSNKALPAPIEKTISKAKGQPREPQVYTLPPSRDELTKNQVSLTCLVKGFYPSDIAVEWESNGQPENNYKTTPPVLDSDGSFFLYSKLTVDKSRWQQGNVFSCSVMHEALHNHYTQKSLSLSPGKGGGGAGGGGGCVLTAIHLNVTDLGLGYETKEELIFRYCSGSCDAAETTYDKILKNLSRNRRLVSDKVGQACCRPIAFDDDLSFLDDNLVYHILRKHSAKRCGCI

SEQ ID NO: 37 - protein, 334 aa, Artificial Sequence
  Synthetic Construct
MEWSWVFLFFLSVTTGVHSAPELLGGPSVFLFPPKPKDTLMISRTPEVTCVVVDVSHEDPEVKFNWYVDGVEVHNAKTKPREEQYNSTYRVVSVLTVLHQDWLNGKEYKCKVSNKALPAPIEKTISKAKGQPREPQVYTLPPSRDELTKNQVSLWCLVKGFYPSDIAVEWESNGQPENNYKTTPPVLDSDGSFFLYSKLTVDKSRWQQGNVFSCSVMHEALHNHYTQKSLSLSPGKGGGGCVLTAIHLNVTDLGLGYETKEELIFRYCSGSCDAAETTYDKILKNLSRNRRLVSDKVGQACCRPIAFDDDLSFLDDNLVYHILRKHSAKRCGCI